European Patent Specification EP 3 638 293 B1, published October 4, 2023. Title: Methods and Compositions for Treating Cancer. Applicant: The University of Chicago. The sequence listing filed with the application follows.

SEQUENCE LISTING (8 sequences)

SEQ ID NO: 1 - protein, 160 aa, Homo sapiens
MVPKLFTSQICLLLLLGLMGVEGSLHARPPQFTRAQWFAIQHISLNPPRCTIAMRAINNYRWRCKNQNTFLRTTFANVVNVCGNQSIRCPHNRTLNNCHRSRFRVPLLHCDLINPGAQNISNCTYADRPGRRFYVVACDNRDPRDSPRYPVVPVHLDTTI

SEQ ID NO: 2 - protein, 267 aa, Homo sapiens
MTLGRRLACLFLACVLPALLLGGTALASEIVGGRRARPHAWPFMVSLQLRGGHFCGATLIAPNFVMSAAHCVANVNVRAVRVVLGAHNLSRREPTRQVFAVQRIFENGYDPVNLLNDIVILQLNGSATINANVQVAQLPAQGRRLGNGVQCLAMGWGLLGRNRGIASVLQELNVTVVTSLCRRSNVCTLVRGRQAGVCFGDSGSPLVCNGLIHGIASFVRGGCASGLYPDAFAPVAQFVNWIDSIIQRSEDNPCPHPRDPDPASRTH

SEQ ID NO: 3 - protein, 255 aa, Homo sapiens
MQPLLLLLAFLLPTGAEAGEIIGGRESRPHSRPYMAYLQIQSPAGQSRCGGFLVREDFVLTAAHCWGSNINVTLGAHNIQRRENTQQHITARRAIRHPQYNQRTIQNDIMLLQLSRRVRRNRNVNPVALPRAQEGLRPGTLCTVAGWGRVSMRRGTDTLREVQLRVQRDRQCLRIFGSYDPRRQICVGDRRERKAAFKGDSGGPLLCNNVAHGIVSYGKSSGVPPEVFTRVSSFLPWIRTTMRSFKLLDQMETPL

SEQ ID NO: 4 - protein, 256 aa, Homo sapiens
MAHRPPSPALASVLLALLLSGAARAAEIVGGHEAQPHSRPYMASLQMRGNPGSHFCGGTLIHPSFVLTAAHCLRDIPQRLVNVVLGAHNVRTQEPTQQHFSVAQVFLNNYDAENKLNDVLLIQLSSPANLSASVATVQLPQQDQPVPHGTQCLAMGWGRVGAHDPPAQVLQELNVTVVTFFCRPHNICTFVPRRKAGICFGDSGGPLICDGIIQGIDSFVIWGCATRLFPDFFTRVALYVDWIRSTLRRVEAKGRP

SEQ ID NO: 5 - protein, 265 aa, Mus musculus
MALGRLSSRTLAAMLLALFLGGPALASEIVGGRPARPHAWPFMASLQRRGGHFCGATLIARNFVMSAAHCVNGLNFRSVQVVLGAHDLRRQERTRQTFSVQRIFENGFDPSQLLNDIVIIQLNGSATINANVQVAQLPAQGQGVGDRTPCLAMGWGRLGTNRPSPSVLQELNVTVVTNMCRRRVNVCTLVPRRQAGICFGDSGGPLVCNNLVQGIDSFIRGGCGSGLYPDAFAPVAEFADWINSIIRSHNDHLLTHPKDREGRTN

SEQ ID NO: 6 - protein, 266 aa, Sus scrofa
MLRLLVVASLVLYGHSTQDFPETNARVVGGTEAQRNSWPSQISLQYRSGSSWAHTCGGTLIRQNWVMTAAHCVDRELTFRVVVGEHNLNQNDGTEQYVGVQKIVVHPYWNTDDVAAGYDIALLRLAQSVTLNSYVQLGVLPRAGTILANNSPCYITGWGLTRTNGQLAQTLQQAYLPTVDYAICSSSSYWGSTVKNSMVCAGGDGVRSGCQGDSGGPLHCLVNGQYAVHGVTSFVSRLGCNVTRKPTVFTRVSAYISWINNVIASN

SEQ ID NO: 7 - protein, 266 aa, Mus musculus
MLRFLVFASLVLCGHSTEDVPETDARVVGGAEARRNSWPSQISLQYQYGGSWHHTCGGTLIRSNWVMTAAHCVDSPMTYRVVVGEHNLSQNDGTEQYVNVQKIVSHPYWNKNNVVAGYDIALLRLAKSVTLNNYVQLGVLPREGTILANNSPCYITGWGRTRTNGELAQTLQQAYLPSVSYSICSSSSYWGSSVKNTMVCAGGDGVRSGCQGDSGGPLHCMVNGQYAVHGVTSFVSSMGCNVARKPTVFTRVSAYISWMNNVIASN

SEQ ID NO: 8 - protein, 269 aa, Rattus norvegicus
MLRFLVFASLVLYGHSTQDFPETNARVVGGAEARRNSWPSQISLQYLSGGSWYHTCGGTLIRRNWVMTAAHCVSSQMTFRVVVGDHNLSQNDGTEQYVSVQKIVVHPNWNSNNVAAGYDIALLRLAQSVTLNNYVQLAVLPQEGTILANNNPCYITGWGRTRTNGQLSQTLQQAYLPSVDYSICSSSSYWGSTVKTTMVCAGGDGVRSGCQGDSGGPLHCLVNGQYSVHGVTSFVSSMGCNVSRKPTVFTRVSAYISWMNNVIAYNSEQ